European Patent Application EP 4 169 381 A1, published April 26, 2023. Title: METHOD FOR INDUCING ENVIRONMENTAL STRESS TOLERANCE OF PLANT. Applicant: Ajinomoto Co., Inc. The sequence listing filed with the application follows.

SEQUENCE LISTING (12 sequences)

SEQ ID NO: 1 - DNA, 20 bp, Artificial Sequence
  primer
aagcggcgcgtggagagaga

SEQ ID NO: 2 - DNA, 20 bp, Artificial Sequence
  primer
gctgtccatctctccgtcgc

SEQ ID NO: 3 - DNA, 21 bp, Artificial Sequence
  primer
tgaagtgatcgatgcaccagg

SEQ ID NO: 4 - DNA, 22 bp, Artificial Sequence
  primer
gacacgacaggaaacacctttg

SEQ ID NO: 5 - DNA, 25 bp, Artificial Sequence
  primer
tatgaatcctctgccgtgagaggtg

SEQ ID NO: 6 - DNA, 24 bp, Artificial Sequence
  primer
acaccactgagataatccgatcct

SEQ ID NO: 7 - DNA, 22 bp, Artificial Sequence
  primer
gttgatggtgtgagtgagcagc

SEQ ID NO: 8 - DNA, 23 bp, Artificial Sequence
  primer
aacccattactagctgtcccaag

SEQ ID NO: 9 - DNA, 22 bp, Artificial Sequence
  primer
accattcagaggttttagcaga

SEQ ID NO: 10 - DNA, 22 bp, Artificial Sequence
  primer
cgttgatgattccacctgattc

SEQ ID NO: 11 - DNA, 21 bp, Artificial Sequence
  primer
ttggtgacaacaggtcaagca

SEQ ID NO: 12 - DNA, 22 bp, Artificial Sequence
  primer
aaacttgtcgctcaatgcaatc